European Patent Specification EP 3 921 440 B1, published March 27, 2024. Title: Method and products for producing functionalised single stranded oligonucleotides. Applicant: Moligo Technologies AB. The sequence listing filed with the application follows.

SEQUENCE LISTING (16 sequences)

SEQ ID NO: 1 - DNA, 378 bp, Artificial Sequence
  Oligonucleotide sequence
ccggcgtcaatacgggataataccgcgccacatagcagaactttaaaagtgctcatcattggaaaacgttcttcggggcgaaaactctcaaggatcttaccgctgttgagatccagttcgatgtaacccactcgtgcacccaactgatcttcagcatcttttactttcaccagcgtttctgggtgagcaaaaacaggaaggcaaaatgccgcaaaaaagggaataagggcgacacggaaatgttgaatactcatactcttcctttttcaatattattgaagcatttatcagggttattgtctcatgagcggatacatatttgaatgtatttagaaaaataaacaaataggggttccgcgcacatttccccgaaaagtg

SEQ ID NO: 2 - DNA, 420 bp, Artificial Sequence
  Oligonucleotide sequence
attgaagcatgcggcgtgcataattctcttactgtcatgccatgcgtaagataccaccacacccgcattcgccattcaggcggccgccaccgcggtggagctccagctgctgtttcctgtgtagagttggtagctcttgatccggtcatatttgttccctttagatccgcctccatctacagggcgcgtccccgcgcttaatgcgcggcctaactacggctacactagaaggacttaccttcggaaaagaaattgttatccgctcacaaaagccagagtatttaagctccctcgtgcgctctcctgttccgggttattgtctcatcggcgaccgagttgctcttgcttatcagaccctgccgcttacaagtggtcgccagtctattaacagcactcaatacgggataatttttcaatatt

SEQ ID NO: 3 - DNA, 78 bp, Artificial Sequence
  Oligonucleotide sequence
gaaccgtcccaagcgttgcgccacatctgctggaaggtggacagtgagaggacacctacgaatcgcaacgggtatcct

SEQ ID NO: 4 - DNA, 77 bp, Artificial Sequence
  Oligonucleotide sequence
gaaccgtcccaagcgttgcgcctgggtacatggtggtaccaccagacaggacacctacgaatcgcaacgggtatcct

SEQ ID NO: 5 - DNA, 76 bp, Artificial Sequence
  Oligonucleotide sequence
gaaccgtcccaagcgttgcggagagcatagccctcgtagatgggcaaggacacctacgaatcgcaacgggtatcct

SEQ ID NO: 6 - DNA, 81 bp, Artificial Sequence
  Oligonucleotide sequence
gaaccgtcccaagcgttgcggtcccagttggtaacaatgccatgttcaatgaggacacctacgaatcgcaacgggtatcct

SEQ ID NO: 7 - DNA, 76 bp, Artificial Sequence
  Oligonucleotide sequence
gaaccgtcccaagcgttgcgcggactcatcgtactcctgcttgctgaggacacctacgaatcgcaacgggtatcct

SEQ ID NO: 8 - DNA, 78 bp, Artificial Sequence
  Oligonucleotide sequence
gaaccgtcccaagcgttgcgttctctttgatgtcacgcacgatttcccaggacacctacgaatcgcaacgggtatcct

SEQ ID NO: 9 - DNA, 80 bp, Artificial Sequence
  Oligonucleotide sequence
gaaccgtcccaagcgttgcgctcggtcaggatcttcatgaggtagtctgtaggacacctacgaatcgcaacgggtatcct

SEQ ID NO: 10 - DNA, 78 bp, Artificial Sequence
  Oligonucleotide sequence
gaaccgtcccaagcgttgcgtttcacggttggccttagggttcaggggaggacacctacgaatcgcaacgggtatcct

SEQ ID NO: 11 - DNA, 78 bp, Artificial Sequence
  Oligonucleotide sequence
gaaccgtcccaagcgttgcggtacttcagggtcaggatacctctcttgaggacacctacgaatcgcaacgggtatcct

SEQ ID NO: 12 - DNA, 79 bp, Artificial Sequence
  Oligonucleotide sequence
gaaccgtcccaagcgttgcgctgctcgaagtctagagcaacatagcacaaggacacctacgaatcgcaacgggtatcct

SEQ ID NO: 13 - DNA, 76 bp, Artificial Sequence
  Oligonucleotide sequence
gaaccgtcccaagcgttgcgcctcgtcacccacataggagtccttcaggacacctacgaatcgcaacgggtatcct

SEQ ID NO: 14 - DNA, 461 bp, Artificial Sequence
  Pseudogene sequence
ggtctcacattgcataattaacatccgcggaacgcggatgttccggcgtcaatacgggataataccgcgccacatagcagaactttaaaagtgctcatcattggaaaacgttcttcggggcgaaaactctcaaggatcttaccgctgttgagatccagttcgatgtaacccactcgtgcacccaactgatcttcagcatcttttactttcaccagcgtttctgggtgagcaaaaacaggaaggcaaaatgccgcaaaaaagggaataagggcgacacggaaatgttgaatactcatactcttcctttttcaatattattgaagcatttatcagggttattgtctcatgagcggatacatatttgaatgtatttagaaaaataaacaaataggggttccgcgcacatttccccgaaaagtgcatccgcggaacgcggatgcagctcttctgcattggagacc

SEQ ID NO: 15 - DNA, 510 bp, Artificial Sequence
  Pseudogene sequence
ggtctcacattgcataaatttcatccgtgggaaccacggatgaaattgaagcatgcggcgtgcataattctcttactgtcatgccatgcgtaagataccaccacacccgcattcgccattcaggcggccgccaccgcggtggagctccagctgctgtttcctgtgtagagttggtagctcttgatccggtcatatttgttccctttagatccgcctccatctacagggcgcgtccccgcgcttaatgcgcggcctaactacggctacactagaaggacttaccttcggaaaagaaattgttatccgctcacaaaagccagagtatttaagctccctcgtgcgctctcctgttccgggttattgtctcatcggcgaccgagttgctcttgcttatcagaccctgccgcttacaagtggtcgccagtctattaacagcactcaatacgggataatttttcaatattcatccgtgggaaccacggatgaatagctcttcatgcattggagacc

SEQ ID NO: 16 - DNA, 1177 bp, Artificial Sequence
  Pseudogene sequence
ggtctcacattgcataatcttcatccgtgggaaccacggatgaagaaccgtcccaagcgttgcgccacatctgctggaaggtggacagtgagaggacacctacgaatcgcaacgggtatcctcatccgtgggaaccacggatgaggaaccgtcccaagcgttgcgcctgggtacatggtggtaccaccagacaggacacctacgaatcgcaacgggtatcctcatccgtgggaaccacggatgaggaaccgtcccaagcgttgcggagagcatagccctcgtagatgggcaaggacacctacgaatcgcaacgggtatcctcatccgtgggaaccacggatgaggaaccgtcccaagcgttgcggtcccagttggtaacaatgccatgttcaatgaggacacctacgaatcgcaacgggtatcctcatccgtgggaaccacggatgaggaaccgtcccaagcgttgcgcggactcatcgtactcctgcttgctgaggacacctacgaatcgcaacgggtatcctcatccgtgggaaccacggatgaggaaccgtcccaagcgttgcgttctctttgatgtcacgcacgatttcccaggacacctacgaatcgcaacgggtatcctcatccgtgggaaccacggatgaggaaccgtcccaagcgttgcgctcggtcaggatcttcatgaggtagtctgtaggacacctacgaatcgcaacgggtatcctcatccgtgggaaccacggatgaggaaccgtcccaagcgttgcgtttcacggttggccttagggttcaggggaggacacctacgaatcgcaacgggtatcctcatccgtgggaaccacggatgaggaaccgtcccaagcgttgcggtacttcagggtcaggatacctctcttgaggacacctacgaatcgcaacgggtatcctcatccgtgggaaccacggatgaggaaccgtcccaagcgttgcgctgctcgaagtctagagcaacatagcacaaggacacctacgaatcgcaacgggtatcctcatccgtgggaaccacggatgaggaaccgtcccaagcgttgcgcctcgtcacccacataggagtccttcaggacacctacgaatcgcaacgggtatcctcatccgtgggaaccacggatgaggagctcttcatgcattggagacc